European Patent Application EP 4 345 108 A1, published April 3, 2024. Title: Cardiac troponin I specific antibody, kit and uses thereof. Applicant: 深圳迈瑞生物医疗电子股份有限公司. The sequence listing filed with the application follows.

SEQUENCE LISTING (30 sequences)

SEQ ID NO: 1 - protein, 5 aa, Artificial sequence
NYAMS

SEQ ID NO: 2 - protein, 17 aa, Artificial sequence
TISSGSSHTFYSDSVKG

SEQ ID NO: 3 - protein, 10 aa, Artificial sequence
ARRWDGAIDY

SEQ ID NO: 4 - protein, 11 aa, Artificial sequence
RASQDISNYLN

SEQ ID NO: 5 - protein, 7 aa, Artificial sequence
YTSRLHS

SEQ ID NO: 6 - protein, 9 aa, Artificial sequence
QQGHTLPLT

SEQ ID NO: 7 - protein, 8 aa, Artificial sequence
GIDLGSFA

SEQ ID NO: 8 - protein, 7 aa, Artificial sequence
INSAGIL

SEQ ID NO: 9 - protein, 6 aa, Artificial sequence
ARLYDL

SEQ ID NO: 10 - protein, 8 aa, Artificial sequence
QSVYDNNA

SEQ ID NO: 11 - protein, 7 aa, Artificial sequence
DASKLAS

SEQ ID NO: 12 - protein, 13 aa, Artificial sequence
LGDYDCSSADCYA

SEQ ID NO: 13 - protein, 8 aa, Artificial sequence
GIDLAGYA

SEQ ID NO: 14 - protein, 7 aa, Artificial sequence
IASDGEK

SEQ ID NO: 15 - protein, 6 aa, Artificial sequence
ARFYDL

SEQ ID NO: 16 - protein, 8 aa, Artificial sequence
ESVYDNNA

SEQ ID NO: 17 - protein, 7 aa, Artificial sequence
DASKVAS

SEQ ID NO: 18 - protein, 13 aa, Artificial sequence
LGDYDCDSGDCYV

SEQ ID NO: 19 - protein, 8 aa, Artificial sequence
GIDLGSFA

SEQ ID NO: 20 - protein, 7 aa, Artificial sequence
INSEDIL

SEQ ID NO: 21 - protein, 6 aa, Artificial sequence
ARFWDL

SEQ ID NO: 22 - protein, 8 aa, Artificial sequence
QSVYDGTA

SEQ ID NO: 23 - protein, 7 aa, Artificial sequence
DASKLAS

SEQ ID NO: 24 - protein, 13 aa, Artificial sequence
LGDYDCSSGDCYV

SEQ ID NO: 25 - protein, 8 aa, Artificial sequence
GYTFTLYV

SEQ ID NO: 26 - protein, 8 aa, Artificial sequence
INPYIDGT

SEQ ID NO: 27 - protein, 15 aa, Artificial sequence
ARSGYGNYGLAWLAY

SEQ ID NO: 28 - protein, 9 aa, Artificial sequence
TGAVTTSNY

SEQ ID NO: 29 - protein, 7 aa, Artificial sequence
GSNNRAP

SEQ ID NO: 30 - protein, 9 aa, Artificial sequence
GLLYSNNWV